European Patent Application EP 4 509 597 A1, published February 19, 2025. Title: 화학적으로 유도된 유도 만능 줄기세포 유래 중간엽 줄기세포로부터 분리된 세포외 소포체 및 이의 용도. Applicant: 인엑소플랫. The sequence listing filed with the application follows.

SEQUENCE LISTING (20 sequences)

SEQ ID NO: 1 - DNA, 22 bp, synthetic construct
  misc_feature 1..22: note = OCT4_Forward Primer
  source 1..22: mol_type = other DNA
cctgaagcagaagaggatcacc

SEQ ID NO: 2 - DNA, 22 bp, synthetic construct
  misc_feature 1..22: note = OCT4_Reverse Primer
  source 1..22: mol_type = other DNA
aaagcggcagatggtcgtttgg

SEQ ID NO: 3 - DNA, 23 bp, synthetic construct
  misc_feature 1..23: note = TBXT_Forward Primer
  source 1..23: mol_type = other DNA
ccttcagcaaagtcaagctcacc

SEQ ID NO: 4 - DNA, 22 bp, synthetic construct
  misc_feature 1..22: note = TBXT_Reverse Primer
  source 1..22: mol_type = other DNA
tgaactgggtctcagggaagca

SEQ ID NO: 5 - DNA, 23 bp, synthetic construct
  misc_feature 1..23: note = SOX17_Forward Primer
  source 1..23: mol_type = other DNA
acgctttcatggtgtgggctaag

SEQ ID NO: 6 - DNA, 21 bp, synthetic construct
  misc_feature 1..21: note = SOX17_Reverse Primer
  source 1..21: mol_type = other DNA
gtcagcgccttccacgacttg

SEQ ID NO: 7 - DNA, 23 bp, synthetic construct
  misc_feature 1..23: note = NCAD_Forward Primer
  source 1..23: mol_type = other DNA
cctccagagtttactgccatgac

SEQ ID NO: 8 - DNA, 22 bp, synthetic construct
  misc_feature 1..22: note = NCAD_Reverse Primer
  source 1..22: mol_type = other DNA
gtaggatctccgccactgattc

SEQ ID NO: 9 - DNA, 23 bp, synthetic construct
  misc_feature 1..23: note = GAPDH_Forward Primer
  source 1..23: mol_type = other DNA
catcactgccacccagaagactg

SEQ ID NO: 10 - DNA, 23 bp, synthetic construct
  misc_feature 1..23: note = GAPDH_Reverse Primer
  source 1..23: mol_type = other DNA
atgccagtgagcttcccgttcag

SEQ ID NO: 11 - DNA, 26 bp, synthetic construct
  misc_feature 1..26: note = IL-1beta_Forward Primer
  source 1..26: mol_type = other DNA
gttcccattagacaactgcactacag

SEQ ID NO: 12 - DNA, 23 bp, synthetic construct
  misc_feature 1..23: note = IL-1beta_Reverse Primer
  source 1..23: mol_type = other DNA
gtcgttgcttggttctccttgta

SEQ ID NO: 13 - DNA, 20 bp, synthetic construct
  misc_feature 1..20: note = TNF-alpha_Forward Primer
  source 1..20: mol_type = other DNA
acggcatggatctcaaagac

SEQ ID NO: 14 - DNA, 20 bp, synthetic construct
  misc_feature 1..20: note = TNF-alpha_Reverse Primer
  source 1..20: mol_type = other DNA
gtgggtgaggagcacgtagt

SEQ ID NO: 15 - DNA, 23 bp, synthetic construct
  misc_feature 1..23: note = IL-6_Forward Primer
  source 1..23: mol_type = other DNA
gaggataccactcccaacagacc

SEQ ID NO: 16 - DNA, 24 bp, synthetic construct
  misc_feature 1..24: note = IL-6_Reverse Primer
  source 1..24: mol_type = other DNA
aagtgcatcatcgttgttcataca

SEQ ID NO: 17 - DNA, 20 bp, synthetic construct
  misc_feature 1..20: note = IL-23_Forward Primer
  source 1..20: mol_type = other DNA
tgcgtgaagggcaaggacac

SEQ ID NO: 18 - DNA, 20 bp, synthetic construct
  misc_feature 1..20: note = IL-23_Reverse Primer
  source 1..20: mol_type = other DNA
aggccaagggctcgagactt

SEQ ID NO: 19 - DNA, 20 bp, synthetic construct
  misc_feature 1..20: note = IL-12b_Forward Primer
  source 1..20: mol_type = other DNA
aggtcacactggaccaaagg

SEQ ID NO: 20 - DNA, 20 bp, synthetic construct
  misc_feature 1..20: note = IL-12b_Reverse Primer
  source 1..20: mol_type = other DNA
tggtttgatgatgtccctag